European Patent Specification EP 3 978 607 B1, published August 20, 2025. Title: Exon-humanized mouse. Applicant: Transgenic Inc. The sequence listing filed with the application follows.

SEQUENCE LISTING (52 sequences)

SEQ ID NO: 1 - DNA, 16913 bp, Artificial
  Synthetic DNA
ctaaattgtaagcgttaatattttgttaaaattcgcgttaaatttttgttaaatcagctcattttttaaccaataggccgaaatcggcaaaatcccttataaatcaaaagaatagaccgagatagggttgagtgttgttccagtttggaacaagagtccactattaaagaacgtggactccaacgtcaaagggcgaaaaaccgtctatcagggcgatggcccactacgtgaaccatcaccctaatcaagttttttggggtcgaggtgccgtaaagcactaaatcggaaccctaaagggagcccccgatttagagcttgacggggaaagccggcgaacgtggcgagaaaggaagggaagaaagcgaaaggagcgggcgctagggcgctggcaagtgtagcggtcacgctgcgcgtaaccaccacacccgccgcgcttaatgcgccgctacagggcgcgtcccattcgccattcaggctgcgcaactgttgggaagggcgatcggtgcgggcctcttcgctattacgccagctggcgaaagggggatgtgctgcaaggcgattaagttgggtaacgccagggttttcccagtcacgacgttgtaaaacgacggccagtgagcgcgcgtaatacgactcactatagggcgaattgggtaccgggccccccctcgaggtcgaccctccaggtcttatccacctcaaggggagctaacaaaattgaattctttgacctgcaaagattcagagccccaaacactgctatttctcttctcctaactcccttaccaggaggcttagtgcaagcatttggcccacctagtccccttcctgctaatcagcttactgcactagcattagcgagcattccagggcctacaaactgctggctaggtgtttgtttggaccttcagaaaacaaatgaagagattgtttaggagatgaaaagatgtattgaacgaggttgtacattttaagggagaaggccgagaagactctctaatcaagagccagccagggttgttcattaactaccataaatttggtagtagggagagagatgtggtcagtaactcaatctctcattcacctaaatgaaacatgtaagctatggcaccgcagccaggatgtgaagaaaaccagtaaagggctaagcaaagacacctccttctaacttaaacactacctccaacacccttatgttctctaggtagttgctgttagtattaccccagaacaggcaatgtcttcagcagaagccccacaaaggcggtgaattttgacacaagtccatccctcatcatggattcctgtaaccatcctctgagaagagtttttacaatttcaactcaatatgtgaaaccacaccttcctttctttagaaaagtatgattgattatccatgggacctattcacagcacaaagtgactcaaaggcaaaaagcacttgggcttctctggggggcaactgccctttatctcacacccatgtcttggacaacaaatgttttcttactctgtctgttttttctgtcctgctctgtcacataaaatcctgcccgacctttgactcaaactccagacagtctacctgctgatcgcccggcccctgttcaaacatgtcctaatactctgtctctgcaagggtcatcagtagttttccatcttactcaacatcctcccagtgcttcaaagcacctcactttatcttcacatccttgtctctttctaattaaagtttaaaaagttggtttctaaggctgatggaggtctaaaaaacaagcaaatcaaagacctgagggtgttctaatttacttggtagttggtcagaactaccagtatgttatggtcagagataaattagggatactatacttagatcaaaatttataaaaagacagagtagagaggatctctgtgagttcaaggttagcctggtcttcgtgcagcgagctccaggctagccaaaggtacaaaatgagattctgtccctaaacagcaaaccaaaaactaaataaaattgataaatgagcatagttcattatgatgaatgctctttacttgtgttagacacagggttgggtgaggcatcacagtgataacagttacagatgcacttagggtatgacactgcctgcagagcacatttgtcaaggaagactaaagccttctggccatgtcctcagggtttacatgaccttatctgaaatgtgtctccagttcaattatctggaatgtgtgtctgcttcagtgcctcacattggtagagaaacattgaccagtgggaggaagccagacaacaaagtcctgggaagagaggattccaggtcctgtgtctgacgaggaatctctcaaagaggtgggcatgcttatttagcaaaagaaaatatgctgtcagaagaccagtaatcataacaaatttataaagaggctgcgctttgtcatggatcgagaatatgggatgtacattaaaaacacacagacaatcagacgtaccagtagtcatgtaatctggcttcagagtgggagagaagtcaggaaaccgagatgtcccaacatgggaccccatagattattttcatgtgaatgtaaggcaactgctgtcatcttccagtttctcaagacaagccaaagtccaggttttaatgcaacgtggttcaatttgcaatttttgcagatatttcaaaatcctagagaaatggtagagcctgtggtcaggtggcagtccagctttgccagtttacgagatcctgggaggcaattcttagtttcaatggattgtggagttcagtagtgtggagttgacatgtgtgggtgagagattttactggatagtgattcctgtatgaagagggctttccatcacattctgagcaatggaaagtaatgatgtcaaccttggttgacaatgcacaagagattctggagaaagcatctccttcttaggcacagatattgaatggaatcatctgacatttgtattttccagtttataaaatgcctttatatcttgtcacatttaaagttcttagaaaatctccttcaaagagaaatgcgatatttctgatttacaaatgtgtggtctgatatctgagataggaaatcatttccagaagcaagcaggacattgagtagcagatctgggattgggtgtgtcagagcctccaacactgtcagactcaaaggtgcaggacaataagtagtcttactctggctgtatcttctcattgttgcttttggacggttgccctctttcccaaaggtgtctgtctgcacatttcgtagagcgagtgttccgatactctaatctccctaggcaaggttcatatttgtgtaggttacttattctccttttgttgactaagtcaataatcagaatcagcaggtttggagtcagcttggcagggatcagcagcctgggttggaaggagggggtataaaagccccttcaccaggagaagccgtcacacagatccacaagctcctgacaggatggcttctcatcgtctgctcctcctctgccttgctggactggtatttgtgtctgaggctggccctacggtgagtgatcctgtgagcgatccagacatggcagttagaccttagataaagaagaagtgccttcttccagatgtgagaactagagtactcagactctatatttaccattagactccaaagagaagagctggagtgcctctggctcttccttctattgctttagcgcattgggtctgtagtgctcagtctctggtgtccttagataataaagatatgagattaacatagaaataaagatataaaagggctggatgtatagtttagtggtccagtgtatgcctagtatgtgaaaagccttctgttcaacctctagcaatagaaaaacaagatatattctcggtggggctgttaatattgaattctcataaaatctttaatatatttagtatgcctattatgttgttatattttagttctttagctaatcaaaatgcattattgatctttctttgtctttttttggccaacactctattccagtctttgaaaaagtcctttaaaagagttaatcagtataattaaatgagtcaggaagtatgtgagggttattttacaaccagagggaattactatagcaacagctgattagaatgatctcaagaaaaagcccattctgtctttttgcaccatgcacctttcagtggctccattcagatggagaggcaaacagagcaatggctctcagagggcctattttccctttgaacattcattatccatatccctggtgcacagcagtgcatctgggggcagaaactgttcttgctttggaaacaatgctgtctatgtcatactggataaagaagctcattaattgtcaacacttatgttatcataatgggatcagcatgtacttttggttttgttccagagtctatcaccggaaagaacaagccggtttactctgacccatttcactgacatttctcttgtctcctctgtgcccagggcaccggtgaatccaagtgtcctctgatggtcaaagttctagatgctgtccgaggcagtcctgccatcaatgtggccgtgcatgtgttcagaaaggctgctgatgacacctgggagccatttgcctctgggtaagcttgtagaaagcccaccatgggaccggttccaggttcccatttgctcttattcgtgttagattcagacacacacaacttaccagctagagggctcagagagagggctcaggggcgaagggcacgtattgctcttgtaagagacacaggtttaattcctagcaccagaatggcagctcataaccatctgaaactcacagtcttaggagatctgggtatctgacattctcttctacccaccatgtgtgtggtgcacaaattcacatgcaggcatcaaatcttataaacaacaacaaaaaaccaacaaacctggtagcaaaagaagattagaaggttaaacatatgagccgagagcttttgttttgttttgttttgttttgttttgtttacatttcaaatgttatcccctttctcggtccccctccccaaaccctctaccccattctctcctccccttcttctatgagggtgttccccaccaacccactcccaccttcctgctctcgaattcccctatactgggacatcaagccttcacagaatcaagggcctctcctcccattgatgcccgacaatgtcatcctctgctacctatgtggctggagccatgggtcccttcatgtatcctccttggttggtggtttagtctctgggaggtctgggggatctggttgattgatattattgttcttcctatgagattgcaaaccccttcagctccttcggtcctttaactcctccactggggaccccgagctcagtccaatggttggctgtgagcatccaccagcagaggcctttttttttttttttaacaaagctgctttattatgttgcttagagcatgaccaggaaccagagcacagtccaagactgaagggaggaaaagggggggagtcaataaccccactgtttcatagtggtttgcaacccttttatatcacagcccactttaggcaaataatgaaaattatagtctccagggacagagaagatggtgcaggaagtgaagtgcctgctcagaaaatgggggcttgaatgtgagttcccagactctgtgtaagatgcccagcatcgaagtgcatgcttataacaccagcctggaggtagaagcttagaaacaggggtaccctgaagttgcttgttcaccagtgtccctgaatgggtaggtgcatgtttggtgagagaccctgtctcaaaaatcaaggtgtaggataattgaaaatacctagctttgagcttagatcatgcaaatgtgtacacacactcacacacaccacacacacaaaaaaatgcagagacagagagatacagagagacagagagatacagagacagagacagagagaaaaggagaaagtaaaaaacaaataatttaaagacccatggccacaaagaggctcaaagacaagcacgtataaaaccatacacatgtaattttaggagttttcagattccctggtacccgtgggtgatgcacaagctttgaatcccagtcttaaaatcttacgaagaacgtgttcgtgtgtgctaatttattgatgagaggaaaggaattgacaaagtgcccttccggagcttcctgcattacccagactcagggtttttttaaatgtacactcagaacagagtagctctgtgcaagggtagcaaccacgaagcttaataagaaacatatcgtgagagatctgcaaggcaaatctaggggctgaccaatctcacagtcacccactagcatgtcaacacaacttcccacctgtgctagccacttagcaattttgtgttgttctgttttgtttttgtttttaacaaagcaatttcaaagagatttctaattcatctaaacaaacaaaccaaaaggaaaacagcaaagacgccctgagcacttagcagagcagctatgcagttatgactcctgggtggagactttatatcaggcttcaactgaatacctagaacctactagtgctcttcatcaatccttgggaaggtcattttcttttggtgctgttttgagtttctatttgttaatgtcttcataattatacacgtgttgagcacagcatgcaaagtgattaggggaatctagttggagtggaatggatacccaaatattcagactttcttgtgactcttctttcttgtacccacatcaaaaaaaaaaaaaatggagatgagacatggtcagagtcactaaaaccagctgctacttttaattacgtggggagcagtttctaacattgccattattgaactgatgctgcctgggtggaaatggaaatcacttagtatttcttgttggcaaagaattactgaatggattaaatttccaaagggagaagtcagttacaagtcttttctttgtttattaggctttctgctatgataaattacactacttccagaagttacccttaggccatgggacactggactatcactctgctgtcacaagagattacagagttagtcaaggcagcttgtgacaccttcagggactgtcataaacttccagcaagtcattaatcctgaatgcaatactgtgtgtgtgtgtctatgtgtgtttgtatgtctgtgtgtgtcttatgtctgtgtctctgtgtgtgtgtgtgtttgtgtgtgtgtgtgtatgtatgcctgtgtgtgtcttatgtctgtgtttgtgtgtctgtgtgtgtcttatgtctgtgtttgtatgtctgtgtgtgtctgtgtgtgtcttatgtctgtgtctctgtgtgtgtgtgtgtgtatgtatgtatgtatgtatgtatgtgtatgtgtttgcatctctctgtgtgtctgcgcttatatatttgtgtatgtgtttatgtgttcgcctttgtgcgttgttggggattgaatccaggggaatacaaatgttaagaaagaacgttaccactaagcttcacctgtaggccttaaagcttttctttcttttaaaaattgtaattaattcattttcagtcaggatctccacacctcgtccctgctgctctagaactcactatttaaacacaatcgccctcaaacctgcagcaaccctcccgcctctaccctgcgagcactagaataataacaggtgaccccacacgcctagattaagacctttaaggtaaacattttactatattttagtctcataagacaagatgctacaataaagctgtacataaagttccctcgaatttcttgctattttaactcaaacataaggatttcctcctttttgattcaggtaacagaaaaaatacacaggtacatacatgtacacacatgaacacacacgcatcacaaccacatatgcgcacgcttgtgtgatctatcatttaccatgccactgaactcttctttccccataaattcctctggacttgtgtgccctccaggaaaaccagtgagtctggagagctgcatgggctcacaactgaggaggaatttgtagaagggatatacaaagtggaaatagacaccaaatcttactggaaggcacttggcatctccccattccatgagcatgcagaggtaagtggacacaccaagttgtttggattttgtttttagtctcaggaaattcccttcgctcttgctgtacgatgggcatgagtggaaagtagattccacagccagaatccacagtgctgggaaagcaagccttctgaatttttctaaaactcatttagcaacatggcctgaacctgttcacactgcttatggtcagctaactatatttatgtaaatattcatttctctgttgaggaaatgttagtatttgcttttgaggcaacctccagataccatggagggcatgtcatagtcaaagagagggctccctatggtatttctctaaattctggcatttcctttattccaaagcacatctagtgtccccagaagtttgggtagacaattcttggcaacacagagaattacaacatgttcaaaacccaacagcttaatatctaaatcatcaagcaaacatcacatggcaaagggatttctgaatcaaaactgtttcatccttatgatcaacctatggaggtctagcctcgacttacacccattttaccaataagctaagagaagctaagttcctcatcaaggacacaaggctagcatgtgtgagcaagtgacagagttgccctctatgttggttagtgtgccttagccagtgtctcagtaagaaatggagctaaatcaaaacccaaggccaacagccaaaggcacatgagtaacctttgcttggcactgggctcagtttccctggctcctctcagtcctcagttcacagaggcagctgtcatgcaaatagaatccaagcttgttggtcagacctggagataacaaattccatcaaaaatagctcctcatgtgacctagtttgctgtctgttgctatgatacacaccatgaccgaaaagcaaccctggggagagaagggtttatttcatcttacagcttacagttcaccatggaggaaagccaggtgggaacctggaagtggaaattgaagcagagaccagaaaggaatgctgtttactggctggcttagctccttttcttatacagcttaggtctatgtgcccaggggatggtactgccgagcataggctgagcccgcctacatcaaccattagtcaaaaaaaggtccatagacttgcctacaggccaatctcatggaggcaataccccagtggagggtccctcttcgcaggttactctagtttgtgtcaagttgacaaaacctaaccacaaagcacaaacagggtctgcccttgtggcttagccatggatgacactctcagatgatggtgttaccagacaaaccagaggggctcaccaagagtctgccacctaccaaggtagtactctactcctcactgggcaccaacacccatattagctgggccagtacaggacccttgctgtttcctgcatgaattgtccatagaccctgggtctcagcctgccgggagtacctgtaagtagtcgcctcaaacacattattcctgttggaagacttgtctgattctcttttagaactcaatcaacaaacgtttttattttgttttggctttttggagacaagatctctcataggccagcctgacttgaatgtagctgaggatgacctgtgctgctaatcttctcgcctcttcctcccaagtggtaggataataggcataagacaccacagcagttttactccataccagggctctgaacccagactttaaacactctatcaactgattcacattcccaccccatcattcaacaaacatttgaaaaataaaacccttctgccttgagcactctgctaaatacagcctttgagtgcggagtatttcctcacaaccagggtccaagatgaccccatcatacataccacggaaaattaggagatgtttttaggtctctttgcttggggtaatttttatgtgtgtgtgtacacagccctgtgcgtgtgtgtgtgtgtgtgtgtgtgtgtgtacaggcacacacgtgtatgcatgtagaggctacataaaaaccttaggtgtcattctcaggcactctgttcaccccttcacacagcccgaacacacaaaatttgaggcattagcctggagctcaccagttaggctagactgacttgccagcagaccccaggctgtctccatctccccagctctgggattacaaactctatcataccagacatttttatacatattctgagcataaaattcatgtcttcaggctaacaagtcaagagcttaaatgactgagctctcttacgtggtggattttttttaaaactacataatatcttttttttttttttcacttctggggaagaaacaaatgagcctgagtgacaatgcgacagaaaagaaattttgaggagtgtgtgtgtctgtgtgtgtggtggcacatgcctctcatctaatgctagaggctacagtagaatgctcctgaattagtggccagccaaggccaagggctagggttgtaactcagtggcagagggcttgcctagcattcgcaggatttgatccatagcgctataaataataataaataaatacaacagtctaagatgattctccctttcatttatctggatgttatttttgtgttagttttactctgtcatccaatcattgtttgccctatatttggacatttaaaaaaaatctttattccaagtgtgttcaaagctgtatccaaaacctgtccaccaaatgagtccaatgacatacatcttctatattaccatctgttccagatttggctgactcccggcacctgggctgttgctgcacccatgtctcagatagtctagtgatttgagaagtgactagtaattgcaaaatccagactttgtccagaaacttctatgagctccaaaactttcatttacatttctgccagccacaaaccgcttgtgttgtggagagaaccctgtgatgtcttcccacagcatctcagccttgtttcttcccttaaaatattcatcttttcacattagaacatgcaaagggacagtgggagcgaaacccctggactgggacgcacgaagccttcctttctggtcaggctctcactgtagaaacttaggccggtttcagcatgcagtctgctggagaatggctcctgccaacattccaggtctggaagtttgtagtggagttgttgataaccactgttcgccacaggtcttttgtttgtgggtgtcagtgtttctactctcctgacttttatctgaacccaagaaagggaacaatagccttcaagctctctgtgactctgatctgaccagggccacccacactgcagaaggaaacttgcaaagagagacctgcaattctctaagagctccacacagctccaaagacttaggcagcatattttaatctaattattcgtcccccaaccccaccccagaggacagttagacaataaaaggaagattaccagcttagcatcctgtgaacactttgtctgcagctcctacctctgggctctgttagaactagctgtctctcctctctcctaggtggtattcacagccaacgactccggcccccgccgctacaccattgccgccctgctgagcccctactcctattccaccacggctgtcgtcaccaatcccaaggaatgagagactcagcccaggaggaccaggatcttgccaaagcagtagcatcccatttgtaccaaaacagtgttcttgctctataaaccgtgttagcagctcaggaagatgccgtgaagcattcttattaaaccacctgctatttcattcaaactgtgtttcttttttatttcctcatttttctcccctgctcctaaaacccaaaatcttctaaagaattctagaaggtatgcgatcaaactttttaaagaaagaaaatactttttgactcatggtttaaaggcatcctttccatcttggggaggtcatgggtgctcctggcaacttgcttgaggaagataggtcagaaagcagagtggaccaaccgttcaatgttttacaagcaaaacatacactaagcatggtctgtagctattaaaagcacacaatctgaagggctgtagatgcacagtagtgttttcccagagcatgttcaaaagccctgggttcaatcacaatactgaaaagtaggccaaaaaacattctgaaaatgaaatatttgggtttttttttataacctttagtgactaaataaagacaaatctaagagactaactgtggctgcttatatcatgttaatttgggtccccaaaattgtttgtatgaacatccacactggtaaataaagttgtggcacccaatggctgggcagggtagatggaggcaggacttttagattcctgggggagggagaaagaaggaggaatcaccatgcctagagaaggagaggagaaacaccatgcctggaaaggtgcgggacagagaacatagccaccatgtaggagcaggaggatagcagccaaagagggctgtacgtctgggtctggggtggccaagagagaatgtaggagttagtaaagtaataactcgggaatatcggagggaggtggattagccacatggaggttaggaagtggcccagccattgagctgattaaagcatatcaaaatataaagaccctgtgcgtgtgtgtgtgtgtgtgtgtgtgtgtgtgtgtgtgtgtgtgtttcatttgagaaccaagaacattcgggcaagtagtgaggaatgagcctcagcaggtgggatctattaaagtatttaattgggtatactacaactgattcttcaggcatttcttgttaagcactttactcatttgagggccataacagtttctttgcacaagaatgggcctatccgcagtcaggcctgggactccgggccccaccccttgctgctgagctatttataatgatacattcaggtagaaggggagtcatggtcttcagttgtgtgctcactggtgactccaccaggctctgatggacagttccaagccaaaatgaagaaacaagccacaaaacgacatgaatctgggagaagggttggtggtaacgtgcggaggggttgggaggtgggaggcagctaagagatgacaaggaagggagcatcagcgtgggctgtgtgcatgcataaaacgaaagcaaacaaaatcaatcactaaaccatgtttaagaacagtgagttccaaagggataaacctgcagcaacccagcttcacttcccaggcaattcctaccttcccatcacagttcatagaacatattcctcctaaactggcaattttccttccagtctttcaaaatgaaataagcttggaatcaattccacttccccagatctctctacccctctaatccactttagaccaattctacctgaatcagaacccagctctcaggagacagaagcagagacaggaggatgtccatgagttcaaggccattctagtgagttctaagccaaccaaaactacataatgagaccttgtctaacaacaacttagtcaaatcctaaatccatgtttaattgatacacacactcatgcacacgcacacacacgtgtaatatgaacaaaacgaaacaaaatagatttgtaatggacgagaataaattcaattttaaccactctgggtttaatataatcagactggtttttaaactctaaagttggcagtgtgtgcacacacatgtccaacgcatggaggtgtgtctcaaaaagcataattataagtattgaactcctacctgcaacatttgatagcacctgtcaaacaaggaaatgaagcatatcttttgcctcaagctatattttatccaccgagcgctcgtagcagaggcagaattatttctccccgatccgtcgtttccccggcgattccttcctttacttcacagtccatagagcttcctaagcgctgttcgttttccctccagcctttcaaaatggaaataagcttagaagcaattccatttccccggctctccattttctctgggtgggagctgccccagttaattttaagccaaagcagatggtaattcatctttggcaaaaccaagtaaatactgaaggtccactctggagcctctgtgagcaagaaggtgggttgcacttggactttctaaaataaaccctagggatgtgcacacagcccccagtgcagcagtcaaccacttgctgttgcttcctcttatttactcccaggaagcaggtggttagagacacgggtacaaggtatgatggaagagaaggcccagacagatgctacaaggtgaacccagaacagctgtcaccatgagaacgtgtgctcagttaaaagaacaacactgctcatctcaggtaacctcaggagctagcatttggaaagcactttagatgtgtttcccagactccagaaaatagcacctaccacacagggcttttaaatgtttgagcatcatatagcatcccttctaagtatgtggaatgaattaatgaatgaaccaatagatgaatgaagtaaaggattagttctaggtaggcaaatctgagccttcgcggccgccaccgcggtggagctccagcttttgttccctttagtgagggttaattgcgcgcttggcgtaatcatggtcatagctgtttcctgtgtgaaattgttatccgctcacaattccacacaacatacgagccggaagcataaagtgtaaagcctggggtgcctaatgagtgagctaactcacattaattgcgttgcgctcactgcccgctttccagtcgggaaacctgtcgtgccagctgcattaatgaatcggccaacgcgcggggagaggcggtttgcgtattgggcgctcttccgcttcctcgctcactgactcgctgcgctcggtcgttcggctgcggcgagcggtatcagctcactcaaaggcggtaatacggttatccacagaatcaggggataacgcaggaaagaacatgtgagcaaaaggccagcaaaaggccaggaaccgtaaaaaggccgcgttgctggcgtttttccataggctccgcccccctgacgagcatcacaaaaatcgacgctcaagtcagaggtggcgaaacccgacaggactataaagataccaggcgtttccccctggaagctccctcgtgcgctctcctgttccgaccctgccgcttaccggatacctgtccgcctttctcccttcgggaagcgtggcgctttctcatagctcacgctgtaggtatctcagttcggtgtaggtcgttcgctccaagctgggctgtgtgcacgaaccccccgttcagcccgaccgctgcgccttatccggtaactatcgtcttgagtccaacccggtaagacacgacttatcgccactggcagcagccactggtaacaggattagcagagcgaggtatgtaggcggtgctacagagttcttgaagtggtggcctaactacggctacactagaaggacagtatttggtatctgcgctctgctgaagccagttaccttcggaaaaagagttggtagctcttgatccggcaaacaaaccaccgctggtagcggtggtttttttgtttgcaagcagcagattacgcgcagaaaaaaaggatctcaagaagatcctttgatcttttctacggggtctgacgctcagtggaacgaaaactcacgttaagggattttggtcatgagattatcaaaaaggatcttcacctagatccttttaaattaaaaatgaagttttaaatcaatctaaagtatatatgagtaaacttggtctgacagttattaccaatgcttaatcagtgaggcacctatctcagcgatctgtctatttcgttcatccatagttgcctgactccccgtcgtgtagataactacgatacgggagggcttaccatctggccccagtgctgcaatgataccgcgagacccacgctcaccggctccagatttatcagcaataaaccagccagccggaagggccgagcgcagaagtggtcctgcaactttatccgcctccatccagtctattaattgttgccgggaagctagagtaagtagttcgccagttaatagtttgcgcaacgttgttgccattgctacaggcatcgtggtgtcacgctcgtcgtttggtatggcttcattcagctccggttcccaacgatcaaggcgagttacatgatcccccatgttgtgcaaaaaagcggttagctccttcggtcctccgatcgttgtcagaagtaagttggccgcagtgttatcactcatggttatggcagcactgcataattctcttactgtcatgccatccgtaagatgcttttctgtgactggtgagtactcaaccaagtcattctgagaatagtgtatgcggcgaccgagttgctcttgcccggcgtcaatacgggataataccgcgccacatagcagaactttaaaagtgctcatcattggaaaacgttcttcggggcgaaaactctcaaggatcttaccgctgttgagatccagttcgatgtaacccactcgtgcacccaactgatcttcagcatcttttactttcaccagcgtttctgggtgagcaaaaacaggaaggcaaaatgccgcaaaaaagggaataagggcgacacggaaatgttgaatactcatactcttcctttttcaatattattgaagcatttatcagggttattgtctcatgagcggatacatatttgaatgtatttagaaaaataaacaaataggggttccgcgcacatttccccgaaaagtgccac

SEQ ID NO: 2 - DNA, 679 bp, Artificial
  Synthetic DNA
ctaaattgtaagcgttaatattttgttaaaattcgcgttaaatttttgttaaatcagctcattttttaaccaataggccgaaatcggcaaaatcccttataaatcaaaagaatagaccgagatagggttgagtgttgttccagtttggaacaagagtccactattaaagaacgtggactccaacgtcaaagggcgaaaaaccgtctatcagggcgatggcccactacgtgaaccatcaccctaatcaagttttttggggtcgaggtgccgtaaagcactaaatcggaaccctaaagggagcccccgatttagagcttgacggggaaagccggcgaacgtggcgagaaaggaagggaagaaagcgaaaggagcgggcgctagggcgctggcaagtgtagcggtcacgctgcgcgtaaccaccacacccgccgcgcttaatgcgccgctacagggcgcgtcccattcgccattcaggctgcgcaactgttgggaagggcgatcggtgcgggcctcttcgctattacgccagctggcgaaagggggatgtgctgcaaggcgattaagttgggtaacgccagggttttcccagtcacgacgttgtaaaacgacggccagtgagcgcgcgtaatacgactcactatagggcgaattgggtaccgggccccccctcgaggtcgac

SEQ ID NO: 3 - DNA, 2621 bp, Mus musculus
cctccaggtcttatccacctcaaggggagctaacaaaattgaattctttgacctgcaaagattcagagccccaaacactgctatttctcttctcctaactcccttaccaggaggcttagtgcaagcatttggcccacctagtccccttcctgctaatcagcttactgcactagcattagcgagcattccagggcctacaaactgctggctaggtgtttgtttggaccttcagaaaacaaatgaagagattgtttaggagatgaaaagatgtattgaacgaggttgtacattttaagggagaaggccgagaagactctctaatcaagagccagccagggttgttcattaactaccataaatttggtagtagggagagagatgtggtcagtaactcaatctctcattcacctaaatgaaacatgtaagctatggcaccgcagccaggatgtgaagaaaaccagtaaagggctaagcaaagacacctccttctaacttaaacactacctccaacacccttatgttctctaggtagttgctgttagtattaccccagaacaggcaatgtcttcagcagaagccccacaaaggcggtgaattttgacacaagtccatccctcatcatggattcctgtaaccatcctctgagaagagtttttacaatttcaactcaatatgtgaaaccacaccttcctttctttagaaaagtatgattgattatccatgggacctattcacagcacaaagtgactcaaaggcaaaaagcacttgggcttctctggggggcaactgccctttatctcacacccatgtcttggacaacaaatgttttcttactctgtctgttttttctgtcctgctctgtcacataaaatcctgcccgacctttgactcaaactccagacagtctacctgctgatcgcccggcccctgttcaaacatgtcctaatactctgtctctgcaagggtcatcagtagttttccatcttactcaacatcctcccagtgcttcaaagcacctcactttatcttcacatccttgtctctttctaattaaagtttaaaaagttggtttctaaggctgatggaggtctaaaaaacaagcaaatcaaagacctgagggtgttctaatttacttggtagttggtcagaactaccagtatgttatggtcagagataaattagggatactatacttagatcaaaatttataaaaagacagagtagagaggatctctgtgagttcaaggttagcctggtcttcgtgcagcgagctccaggctagccaaaggtacaaaatgagattctgtccctaaacagcaaaccaaaaactaaataaaattgataaatgagcatagttcattatgatgaatgctctttacttgtgttagacacagggttgggtgaggcatcacagtgataacagttacagatgcacttagggtatgacactgcctgcagagcacatttgtcaaggaagactaaagccttctggccatgtcctcagggtttacatgaccttatctgaaatgtgtctccagttcaattatctggaatgtgtgtctgcttcagtgcctcacattggtagagaaacattgaccagtgggaggaagccagacaacaaagtcctgggaagagaggattccaggtcctgtgtctgacgaggaatctctcaaagaggtgggcatgcttatttagcaaaagaaaatatgctgtcagaagaccagtaatcataacaaatttataaagaggctgcgctttgtcatggatcgagaatatgggatgtacattaaaaacacacagacaatcagacgtaccagtagtcatgtaatctggcttcagagtgggagagaagtcaggaaaccgagatgtcccaacatgggaccccatagattattttcatgtgaatgtaaggcaactgctgtcatcttccagtttctcaagacaagccaaagtccaggttttaatgcaacgtggttcaatttgcaatttttgcagatatttcaaaatcctagagaaatggtagagcctgtggtcaggtggcagtccagctttgccagtttacgagatcctgggaggcaattcttagtttcaatggattgtggagttcagtagtgtggagttgacatgtgtgggtgagagattttactggatagtgattcctgtatgaagagggctttccatcacattctgagcaatggaaagtaatgatgtcaaccttggttgacaatgcacaagagattctggagaaagcatctccttcttaggcacagatattgaatggaatcatctgacatttgtattttccagtttataaaatgcctttatatcttgtcacatttaaagttcttagaaaatctccttcaaagagaaatgcgatatttctgatttacaaatgtgtggtctgatatctgagataggaaatcatttccagaagcaagcaggacattgagtagcagatctgggattgggtgtgtcagagcctccaacactgtcagactcaaaggtgcaggacaataagtagtcttactctggctgtatcttctcattgttgcttttggacggttgccctctttcccaaaggtgtctgtctgcacatttcgtagagcgagtgttccgatact

SEQ ID NO: 4 - DNA, 258 bp, Homo sapiens
ctaatctccctaggcaaggttcatatttgtgtaggttacttattctccttttgttgactaagtcaataatcagaatcagcaggtttggagtcagcttggcagggatcagcagcctgggttggaaggagggggtataaaagccccttcaccaggagaagccgtcacacagatccacaagctcctgacaggatggcttctcatcgtctgctcctcctctgccttgctggactggtatttgtgtctgaggctggccctacg

SEQ ID NO: 5 - DNA, 948 bp, Mus musculus
gtgagtgatcctgtgagcgatccagacatggcagttagaccttagataaagaagaagtgccttcttccagatgtgagaactagagtactcagactctatatttaccattagactccaaagagaagagctggagtgcctctggctcttccttctattgctttagcgcattgggtctgtagtgctcagtctctggtgtccttagataataaagatatgagattaacatagaaataaagatataaaagggctggatgtatagtttagtggtccagtgtatgcctagtatgtgaaaagccttctgttcaacctctagcaatagaaaaacaagatatattctcggtggggctgttaatattgaattctcataaaatctttaatatatttagtatgcctattatgttgttatattttagttctttagctaatcaaaatgcattattgatctttctttgtctttttttggccaacactctattccagtctttgaaaaagtcctttaaaagagttaatcagtataattaaatgagtcaggaagtatgtgagggttattttacaaccagagggaattactatagcaacagctgattagaatgatctcaagaaaaagcccattctgtctttttgcaccatgcacctttcagtggctccattcagatggagaggcaaacagagcaatggctctcagagggcctattttccctttgaacattcattatccatatccctggtgcacagcagtgcatctgggggcagaaactgttcttgctttggaaacaatgctgtctatgtcatactggataaagaagctcattaattgtcaacacttatgttatcataatgggatcagcatgtacttttggttttgttccagagtctatcaccggaaagaacaagccggtttactctgacccatttcactgacatttctcttgtctcctctgtgcccag

SEQ ID NO: 6 - DNA, 131 bp, Homo sapiens
ggcaccggtgaatccaagtgtcctctgatggtcaaagttctagatgctgtccgaggcagtcctgccatcaatgtggccgtgcatgtgttcagaaaggctgctgatgacacctgggagccatttgcctctgg

SEQ ID NO: 7 - DNA, 3392 bp, Mus musculus
gtaagcttgtagaaagcccaccatgggaccggttccaggttcccatttgctcttattcgtgttagattcagacacacacaacttaccagctagagggctcagagagagggctcaggggcgaagggcacgtattgctcttgtaagagacacaggtttaattcctagcaccagaatggcagctcataaccatctgaaactcacagtcttaggagatctgggtatctgacattctcttctacccaccatgtgtgtggtgcacaaattcacatgcaggcatcaaatcttataaacaacaacaaaaaaccaacaaacctggtagcaaaagaagattagaaggttaaacatatgagccgagagcttttgttttgttttgttttgttttgttttgtttacatttcaaatgttatcccctttctcggtccccctccccaaaccctctaccccattctctcctccccttcttctatgagggtgttccccaccaacccactcccaccttcctgctctcgaattcccctatactgggacatcaagccttcacagaatcaagggcctctcctcccattgatgcccgacaatgtcatcctctgctacctatgtggctggagccatgggtcccttcatgtatcctccttggttggtggtttagtctctgggaggtctgggggatctggttgattgatattattgttcttcctatgagattgcaaaccccttcagctccttcggtcctttaactcctccactggggaccccgagctcagtccaatggttggctgtgagcatccaccagcagaggcctttttttttttttttaacaaagctgctttattatgttgcttagagcatgaccaggaaccagagcacagtccaagactgaagggaggaaaagggggggagtcaataaccccactgtttcatagtggtttgcaacccttttatatcacagcccactttaggcaaataatgaaaattatagtctccagggacagagaagatggtgcaggaagtgaagtgcctgctcagaaaatgggggcttgaatgtgagttcccagactctgtgtaagatgcccagcatcgaagtgcatgcttataacaccagcctggaggtagaagcttagaaacaggggtaccctgaagttgcttgttcaccagtgtccctgaatgggtaggtgcatgtttggtgagagaccctgtctcaaaaatcaaggtgtaggataattgaaaatacctagctttgagcttagatcatgcaaatgtgtacacacactcacacacaccacacacacaaaaaaatgcagagacagagagatacagagagacagagagatacagagacagagacagagagaaaaggagaaagtaaaaaacaaataatttaaagacccatggccacaaagaggctcaaagacaagcacgtataaaaccatacacatgtaattttaggagttttcagattccctggtacccgtgggtgatgcacaagctttgaatcccagtcttaaaatcttacgaagaacgtgttcgtgtgtgctaatttattgatgagaggaaaggaattgacaaagtgcccttccggagcttcctgcattacccagactcagggtttttttaaatgtacactcagaacagagtagctctgtgcaagggtagcaaccacgaagcttaataagaaacatatcgtgagagatctgcaaggcaaatctaggggctgaccaatctcacagtcacccactagcatgtcaacacaacttcccacctgtgctagccacttagcaattttgtgttgttctgttttgtttttgtttttaacaaagcaatttcaaagagatttctaattcatctaaacaaacaaaccaaaaggaaaacagcaaagacgccctgagcacttagcagagcagctatgcagttatgactcctgggtggagactttatatcaggcttcaactgaatacctagaacctactagtgctcttcatcaatccttgggaaggtcattttcttttggtgctgttttgagtttctatttgttaatgtcttcataattatacacgtgttgagcacagcatgcaaagtgattaggggaatctagttggagtggaatggatacccaaatattcagactttcttgtgactcttctttcttgtacccacatcaaaaaaaaaaaaaatggagatgagacatggtcagagtcactaaaaccagctgctacttttaattacgtggggagcagtttctaacattgccattattgaactgatgctgcctgggtggaaatggaaatcacttagtatttcttgttggcaaagaattactgaatggattaaatttccaaagggagaagtcagttacaagtcttttctttgtttattaggctttctgctatgataaattacactacttccagaagttacccttaggccatgggacactggactatcactctgctgtcacaagagattacagagttagtcaaggcagcttgtgacaccttcagggactgtcataaacttccagcaagtcattaatcctgaatgcaatactgtgtgtgtgtgtctatgtgtgtttgtatgtctgtgtgtgtcttatgtctgtgtctctgtgtgtgtgtgtgtttgtgtgtgtgtgtgtatgtatgcctgtgtgtgtcttatgtctgtgtttgtgtgtctgtgtgtgtcttatgtctgtgtttgtatgtctgtgtgtgtctgtgtgtgtcttatgtctgtgtctctgtgtgtgtgtgtgtgtatgtatgtatgtatgtatgtatgtgtatgtgtttgcatctctctgtgtgtctgcgcttatatatttgtgtatgtgtttatgtgttcgcctttgtgcgttgttggggattgaatccaggggaatacaaatgttaagaaagaacgttaccactaagcttcacctgtaggccttaaagcttttctttcttttaaaaattgtaattaattcattttcagtcaggatctccacacctcgtccctgctgctctagaactcactatttaaacacaatcgccctcaaacctgcagcaaccctcccgcctctaccctgcgagcactagaataataacaggtgaccccacacgcctagattaagacctttaaggtaaacattttactatattttagtctcataagacaagatgctacaataaagctgtacataaagttccctcgaatttcttgctattttaactcaaacataaggatttcctcctttttgattcaggtaacagaaaaaatacacaggtacatacatgtacacacatgaacacacacgcatcacaaccacatatgcgcacgcttgtgtgatctatcatttaccatgccactgaactcttctttccccataaattcctctggacttgtgtgccctccag

SEQ ID NO: 8 - DNA, 136 bp, Homo sapiens
gaaaaccagtgagtctggagagctgcatgggctcacaactgaggaggaatttgtagaagggatatacaaagtggaaatagacaccaaatcttactggaaggcacttggcatctccccattccatgagcatgcagag

SEQ ID NO: 9 - DNA, 3516 bp, Mus musculus
gtaagtggacacaccaagttgtttggattttgtttttagtctcaggaaattcccttcgctcttgctgtacgatgggcatgagtggaaagtagattccacagccagaatccacagtgctgggaaagcaagccttctgaatttttctaaaactcatttagcaacatggcctgaacctgttcacactgcttatggtcagctaactatatttatgtaaatattcatttctctgttgaggaaatgttagtatttgcttttgaggcaacctccagataccatggagggcatgtcatagtcaaagagagggctccctatggtatttctctaaattctggcatttcctttattccaaagcacatctagtgtccccagaagtttgggtagacaattcttggcaacacagagaattacaacatgttcaaaacccaacagcttaatatctaaatcatcaagcaaacatcacatggcaaagggatttctgaatcaaaactgtttcatccttatgatcaacctatggaggtctagcctcgacttacacccattttaccaataagctaagagaagctaagttcctcatcaaggacacaaggctagcatgtgtgagcaagtgacagagttgccctctatgttggttagtgtgccttagccagtgtctcagtaagaaatggagctaaatcaaaacccaaggccaacagccaaaggcacatgagtaacctttgcttggcactgggctcagtttccctggctcctctcagtcctcagttcacagaggcagctgtcatgcaaatagaatccaagcttgttggtcagacctggagataacaaattccatcaaaaatagctcctcatgtgacctagtttgctgtctgttgctatgatacacaccatgaccgaaaagcaaccctggggagagaagggtttatttcatcttacagcttacagttcaccatggaggaaagccaggtgggaacctggaagtggaaattgaagcagagaccagaaaggaatgctgtttactggctggcttagctccttttcttatacagcttaggtctatgtgcccaggggatggtactgccgagcataggctgagcccgcctacatcaaccattagtcaaaaaaaggtccatagacttgcctacaggccaatctcatggaggcaataccccagtggagggtccctcttcgcaggttactctagtttgtgtcaagttgacaaaacctaaccacaaagcacaaacagggtctgcccttgtggcttagccatggatgacactctcagatgatggtgttaccagacaaaccagaggggctcaccaagagtctgccacctaccaaggtagtactctactcctcactgggcaccaacacccatattagctgggccagtacaggacccttgctgtttcctgcatgaattgtccatagaccctgggtctcagcctgccgggagtacctgtaagtagtcgcctcaaacacattattcctgttggaagacttgtctgattctcttttagaactcaatcaacaaacgtttttattttgttttggctttttggagacaagatctctcataggccagcctgacttgaatgtagctgaggatgacctgtgctgctaatcttctcgcctcttcctcccaagtggtaggataataggcataagacaccacagcagttttactccataccagggctctgaacccagactttaaacactctatcaactgattcacattcccaccccatcattcaacaaacatttgaaaaataaaacccttctgccttgagcactctgctaaatacagcctttgagtgcggagtatttcctcacaaccagggtccaagatgaccccatcatacataccacggaaaattaggagatgtttttaggtctctttgcttggggtaatttttatgtgtgtgtgtacacagccctgtgcgtgtgtgtgtgtgtgtgtgtgtgtgtgtacaggcacacacgtgtatgcatgtagaggctacataaaaaccttaggtgtcattctcaggcactctgttcaccccttcacacagcccgaacacacaaaatttgaggcattagcctggagctcaccagttaggctagactgacttgccagcagaccccaggctgtctccatctccccagctctgggattacaaactctatcataccagacatttttatacatattctgagcataaaattcatgtcttcaggctaacaagtcaagagcttaaatgactgagctctcttacgtggtggattttttttaaaactacataatatcttttttttttttttcacttctggggaagaaacaaatgagcctgagtgacaatgcgacagaaaagaaattttgaggagtgtgtgtgtctgtgtgtgtggtggcacatgcctctcatctaatgctagaggctacagtagaatgctcctgaattagtggccagccaaggccaagggctagggttgtaactcagtggcagagggcttgcctagcattcgcaggatttgatccatagcgctataaataataataaataaatacaacagtctaagatgattctccctttcatttatctggatgttatttttgtgttagttttactctgtcatccaatcattgtttgccctatatttggacatttaaaaaaaatctttattccaagtgtgttcaaagctgtatccaaaacctgtccaccaaatgagtccaatgacatacatcttctatattaccatctgttccagatttggctgactcccggcacctgggctgttgctgcacccatgtctcagatagtctagtgatttgagaagtgactagtaattgcaaaatccagactttgtccagaaacttctatgagctccaaaactttcatttacatttctgccagccacaaaccgcttgtgttgtggagagaaccctgtgatgtcttcccacagcatctcagccttgtttcttcccttaaaatattcatcttttcacattagaacatgcaaagggacagtgggagcgaaacccctggactgggacgcacgaagccttcctttctggtcaggctctcactgtagaaacttaggccggtttcagcatgcagtctgctggagaatggctcctgccaacattccaggtctggaagtttgtagtggagttgttgataaccactgttcgccacaggtcttttgtttgtgggtgtcagtgtttctactctcctgacttttatctgaacccaagaaagggaacaatagccttcaagctctctgtgactctgatctgaccagggccacccacactgcagaaggaaacttgcaaagagagacctgcaattctctaagagctccacacagctccaaagacttaggcagcatattttaatctaattattcgtcccccaaccccaccccagaggacagttagacaataaaaggaagattaccagcttagcatcctgtgaacactttgtctgcagctcctacctctgggctctgttagaactagctgtctctcctctctcctag

SEQ ID NO: 10 - DNA, 696 bp, Homo sapiens
gtggtattcacagccaacgactccggcccccgccgctacaccattgccgccctgctgagcccctactcctattccaccacggctgtcgtcaccaatcccaaggaatgagagactcagcccaggaggaccaggatcttgccaaagcagtagcatcccatttgtaccaaaacagtgttcttgctctataaaccgtgttagcagctcaggaagatgccgtgaagcattcttattaaaccacctgctatttcattcaaactgtgtttcttttttatttcctcatttttctcccctgctcctaaaacccaaaatcttctaaagaattctagaaggtatgcgatcaaactttttaaagaaagaaaatactttttgactcatggtttaaaggcatcctttccatcttggggaggtcatgggtgctcctggcaacttgcttgaggaagataggtcagaaagcagagtggaccaaccgttcaatgttttacaagcaaaacatacactaagcatggtctgtagctattaaaagcacacaatctgaagggctgtagatgcacagtagtgttttcccagagcatgttcaaaagccctgggttcaatcacaatactgaaaagtaggccaaaaaacattctgaaaatgaaatatttgggtttttttttataacctttagtgactaaataaagacaaatctaagagactaa

SEQ ID NO: 11 - DNA, 2308 bp, Mus musculus
ctgtggctgcttatatcatgttaatttgggtccccaaaattgtttgtatgaacatccacactggtaaataaagttgtggcacccaatggctgggcagggtagatggaggcaggacttttagattcctgggggagggagaaagaaggaggaatcaccatgcctagagaaggagaggagaaacaccatgcctggaaaggtgcgggacagagaacatagccaccatgtaggagcaggaggatagcagccaaagagggctgtacgtctgggtctggggtggccaagagagaatgtaggagttagtaaagtaataactcgggaatatcggagggaggtggattagccacatggaggttaggaagtggcccagccattgagctgattaaagcatatcaaaatataaagaccctgtgcgtgtgtgtgtgtgtgtgtgtgtgtgtgtgtgtgtgtgtgtgtttcatttgagaaccaagaacattcgggcaagtagtgaggaatgagcctcagcaggtgggatctattaaagtatttaattgggtatactacaactgattcttcaggcatttcttgttaagcactttactcatttgagggccataacagtttctttgcacaagaatgggcctatccgcagtcaggcctgggactccgggccccaccccttgctgctgagctatttataatgatacattcaggtagaaggggagtcatggtcttcagttgtgtgctcactggtgactccaccaggctctgatggacagttccaagccaaaatgaagaaacaagccacaaaacgacatgaatctgggagaagggttggtggtaacgtgcggaggggttgggaggtgggaggcagctaagagatgacaaggaagggagcatcagcgtgggctgtgtgcatgcataaaacgaaagcaaacaaaatcaatcactaaaccatgtttaagaacagtgagttccaaagggataaacctgcagcaacccagcttcacttcccaggcaattcctaccttcccatcacagttcatagaacatattcctcctaaactggcaattttccttccagtctttcaaaatgaaataagcttggaatcaattccacttccccagatctctctacccctctaatccactttagaccaattctacctgaatcagaacccagctctcaggagacagaagcagagacaggaggatgtccatgagttcaaggccattctagtgagttctaagccaaccaaaactacataatgagaccttgtctaacaacaacttagtcaaatcctaaatccatgtttaattgatacacacactcatgcacacgcacacacacgtgtaatatgaacaaaacgaaacaaaatagatttgtaatggacgagaataaattcaattttaaccactctgggtttaatataatcagactggtttttaaactctaaagttggcagtgtgtgcacacacatgtccaacgcatggaggtgtgtctcaaaaagcataattataagtattgaactcctacctgcaacatttgatagcacctgtcaaacaaggaaatgaagcatatcttttgcctcaagctatattttatccaccgagcgctcgtagcagaggcagaattatttctccccgatccgtcgtttccccggcgattccttcctttacttcacagtccatagagcttcctaagcgctgttcgttttccctccagcctttcaaaatggaaataagcttagaagcaattccatttccccggctctccattttctctgggtgggagctgccccagttaattttaagccaaagcagatggtaattcatctttggcaaaaccaagtaaatactgaaggtccactctggagcctctgtgagcaagaaggtgggttgcacttggactttctaaaataaaccctagggatgtgcacacagcccccagtgcagcagtcaaccacttgctgttgcttcctcttatttactcccaggaagcaggtggttagagacacgggtacaaggtatgatggaagagaaggcccagacagatgctacaaggtgaacccagaacagctgtcaccatgagaacgtgtgctcagttaaaagaacaacactgctcatctcaggtaacctcaggagctagcatttggaaagcactttagatgtgtttcccagactccagaaaatagcacctaccacacagggcttttaaatgtttgagcatcatatagcatcccttctaagtatgtggaatgaattaatgaatgaaccaatagatgaatgaagtaaaggattagttctaggtaggcaaatctgagccttc

SEQ ID NO: 12 - DNA, 2228 bp, Artificial
  Synthetic DNA
gcggccgccaccgcggtggagctccagcttttgttccctttagtgagggttaattgcgcgcttggcgtaatcatggtcatagctgtttcctgtgtgaaattgttatccgctcacaattccacacaacatacgagccggaagcataaagtgtaaagcctggggtgcctaatgagtgagctaactcacattaattgcgttgcgctcactgcccgctttccagtcgggaaacctgtcgtgccagctgcattaatgaatcggccaacgcgcggggagaggcggtttgcgtattgggcgctcttccgcttcctcgctcactgactcgctgcgctcggtcgttcggctgcggcgagcggtatcagctcactcaaaggcggtaatacggttatccacagaatcaggggataacgcaggaaagaacatgtgagcaaaaggccagcaaaaggccaggaaccgtaaaaaggccgcgttgctggcgtttttccataggctccgcccccctgacgagcatcacaaaaatcgacgctcaagtcagaggtggcgaaacccgacaggactataaagataccaggcgtttccccctggaagctccctcgtgcgctctcctgttccgaccctgccgcttaccggatacctgtccgcctttctcccttcgggaagcgtggcgctttctcatagctcacgctgtaggtatctcagttcggtgtaggtcgttcgctccaagctgggctgtgtgcacgaaccccccgttcagcccgaccgctgcgccttatccggtaactatcgtcttgagtccaacccggtaagacacgacttatcgccactggcagcagccactggtaacaggattagcagagcgaggtatgtaggcggtgctacagagttcttgaagtggtggcctaactacggctacactagaaggacagtatttggtatctgcgctctgctgaagccagttaccttcggaaaaagagttggtagctcttgatccggcaaacaaaccaccgctggtagcggtggtttttttgtttgcaagcagcagattacgcgcagaaaaaaaggatctcaagaagatcctttgatcttttctacggggtctgacgctcagtggaacgaaaactcacgttaagggattttggtcatgagattatcaaaaaggatcttcacctagatccttttaaattaaaaatgaagttttaaatcaatctaaagtatatatgagtaaacttggtctgacagttattaccaatgcttaatcagtgaggcacctatctcagcgatctgtctatttcgttcatccatagttgcctgactccccgtcgtgtagataactacgatacgggagggcttaccatctggccccagtgctgcaatgataccgcgagacccacgctcaccggctccagatttatcagcaataaaccagccagccggaagggccgagcgcagaagtggtcctgcaactttatccgcctccatccagtctattaattgttgccgggaagctagagtaagtagttcgccagttaatagtttgcgcaacgttgttgccattgctacaggcatcgtggtgtcacgctcgtcgtttggtatggcttcattcagctccggttcccaacgatcaaggcgagttacatgatcccccatgttgtgcaaaaaagcggttagctccttcggtcctccgatcgttgtcagaagtaagttggccgcagtgttatcactcatggttatggcagcactgcataattctcttactgtcatgccatccgtaagatgcttttctgtgactggtgagtactcaaccaagtcattctgagaatagtgtatgcggcgaccgagttgctcttgcccggcgtcaatacgggataataccgcgccacatagcagaactttaaaagtgctcatcattggaaaacgttcttcggggcgaaaactctcaaggatcttaccgctgttgagatccagttcgatgtaacccactcgtgcacccaactgatcttcagcatcttttactttcaccagcgtttctgggtgagcaaaaacaggaaggcaaaatgccgcaaaaaagggaataagggcgacacggaaatgttgaatactcatactcttcctttttcaatattattgaagcatttatcagggttattgtctcatgagcggatacatatttgaatgtatttagaaaaataaacaaataggggttccgcgcacatttccccgaaaagtgccac

SEQ ID NO: 13 - DNA, 23 bp, Artificial
  Synthetic DNA
ctgctcctcctctgccttgctgg

SEQ ID NO: 14 - DNA, 23 bp, Artificial
  Synthetic DNA
gcagaggaggagcagacgatgag

SEQ ID NO: 15 - DNA, 48 bp, Artificial
  Synthetic DNA
caccctgctcctcctctgccttgcgacgaggaggagacggaacgcaaa

SEQ ID NO: 16 - DNA, 48 bp, Artificial
  Synthetic DNA
caccgcaaaggaggaagagtcgaacgtttcctccttctcagcttcaaa

SEQ ID NO: 17 - DNA, 23 bp, Artificial
  Synthetic DNA
ctgcgatggtgtagtggcgatgg

SEQ ID NO: 18 - DNA, 23 bp, Artificial
  Synthetic DNA
gtggcgatggccagagtcgttgg

SEQ ID NO: 19 - DNA, 48 bp, Artificial
  Synthetic DNA
caccctgcgatggtgtagtggcgagacgctaccacatcaccgctcaaa

SEQ ID NO: 20 - DNA, 48 bp, Artificial
  Synthetic DNA
caccgtggcgatggccagagtcgtcaccgctaccggtctcagcacaaa

SEQ ID NO: 21 - DNA, 24 bp, Artificial
  Synthetic DNA
ggattgtggagttcagtagtgtgg

SEQ ID NO: 22 - DNA, 19 bp, Artificial
  Synthetic DNA
ctgagcaggcacttcactt

SEQ ID NO: 23 - DNA, 26 bp, Artificial
  Synthetic DNA
agcgagtgttccgatactctaatctc

SEQ ID NO: 24 - DNA, 24 bp, Artificial
  Synthetic DNA
atggctctcagagggcctattttc

SEQ ID NO: 25 - DNA, 97 bp, Mus musculus
aagctcctgacaggatggcttcccttcgactcttcctcctttgcctcgctggactggtatttgtgtctgaagctggccccgcggtgagtgatcctgt

SEQ ID NO: 26 - DNA, 97 bp, Homo sapiens
aagctcctgacaggatggcttctcatcgtctgctcctcctctgccttgctggactggtatttgtgtctgaggctggccctacggtgagtgatcctgt

SEQ ID NO: 27 - DNA, 131 bp, Mus musculus
ggtgctggagaatccaaatgtcctctgatggtcaaagtcctggatgctgtccgaggcagccctgctgtagacgtggctgtaaaagtgttcaaaaagacctctgagggatcctgggagccctttgcctctgg

SEQ ID NO: 28 - DNA, 131 bp, Homo sapiens; identical to SEQ ID NO: 6

SEQ ID NO: 29 - DNA, 23 bp, Artificial
  Synthetic DNA
aacaggtgaccccacacgcctag

SEQ ID NO: 30 - DNA, 20 bp, Artificial
  Synthetic DNA
actggctaaggcacactaac

SEQ ID NO: 31 - DNA, 25 bp, Artificial
  Synthetic DNA
tatgcgcacgcttgtgtgatctatc

SEQ ID NO: 32 - DNA, 135 bp, Mus musculus
aagaccgcggagtctggagagctgcacgggctcaccacagatgagaagtttgtagaaggagtgtacagagtagaactggacaccaaatcgtactggaagacacttggcatttccccgttccatgaattcgcggat

SEQ ID NO: 33 - DNA, 135 bp, Homo sapiens
aaaaccagtgagtctggagagctgcatgggctcacaactgaggaggaatttgtagaagggatatacaaagtggaaatagacaccaaatcttactggaaggcacttggcatctccccattccatgagcatgcagag

SEQ ID NO: 34 - DNA, 20 bp, Artificial
  Synthetic DNA
gtatccaaaacctgtccacc

SEQ ID NO: 35 - DNA, 22 bp, Artificial
  Synthetic DNA
gcagccacagttagtctcttag

SEQ ID NO: 36 - DNA, 23 bp, Artificial
  Synthetic DNA
ccacacagctccaaagacttagg

SEQ ID NO: 37 - DNA, 108 bp, Mus musculus
gtggttttcacagccaacgactctggccatcgccactacaccatcgcagccctgctcagcccatactcctacagcaccacggctgtcgtcagcaacccccagaattga

SEQ ID NO: 38 - DNA, 108 bp, Homo sapiens
gtggtattcacagccaacgactccggcccccgccgctacaccattgccgccctgctgagcccctactcctattccaccacggctgtcgtcaccaatcccaaggaatga

SEQ ID NO: 39 - DNA, 25 bp, Artificial
  Synthetic DNA
ctaatctccctaggcaaggttcata

SEQ ID NO: 40 - DNA, 25 bp, Artificial
  Synthetic DNA
aagccatcctgtcaggagcttgtgg

SEQ ID NO: 41 - DNA, 23 bp, Artificial
  Synthetic DNA
ggtcagaaggactcctatgtggg

SEQ ID NO: 42 - DNA, 20 bp, Artificial
  Synthetic DNA
atgaggtagtctgtcaggtc

SEQ ID NO: 43 - DNA, 52 bp, Artificial
  Synthetic DNA
ggcaccggtgaatccaagtgtcctctgatggtcaaagttctagatgctgtcc

SEQ ID NO: 44 - DNA, 23 bp, Artificial
  Synthetic DNA
tgaatccaagtgtcctctgatgg

SEQ ID NO: 45 - DNA, 42 bp, Artificial
  Synthetic DNA/RNA
tgaatccaagtgtcctctgaguuuuagagcuaugcuguuuug

SEQ ID NO: 46 - RNA, 69 nt, Artificial
  Synthetic DNA
aaacagcauagcaaguuaaaauaaggcuaguccguuaucaacuugaaaaaguggcaccgagucggugcu

SEQ ID NO: 47 - DNA, 123 bp, Artificial
  Synthetic DNA
tgacccatttcactgacatttctcttgtctcctctgtgcccagggcaccggtgaatccaaatgtcctctgatggtcaaagttctagatgctgtccgaggcagtcctgccatcaatgtggccgt

SEQ ID NO: 48 - DNA, 23 bp, Artificial
  Synthetic DNA
tccactcattcttggcaggatgg

SEQ ID NO: 49 - DNA, 19 bp, Artificial
  Synthetic DNA
ctcattcttggcaggatgg

SEQ ID NO: 50 - DNA, 40 bp, Artificial
  Synthetic DNA
caccctcattcttggcaggagagtaagaaccgtcctcaaa

SEQ ID NO: 51 - DNA, 23 bp, Artificial
  Synthetic DNA
tgaatccaaatgtcctctgatgg

SEQ ID NO: 52 - DNA, 48 bp, Artificial
  Synthetic DNA
cacctgaatccaaatgtcctctgaaggtgagtaagaaccgtcctcaaa